European Patent Specification EP 3 538 101 B1, published June 19, 2024. Title: Inhibitors of Cancer Invasion, Attachment, and/or Metastasis. Applicant: Virginia Commonwealth University Fisher, Paul B. Pellecchia, Maurizio Das, Swadesh K. Kegelman, Timothy P. Wu, Bainan De, Surya K. Wei, Jun Menezes, Mitchell E. Emdad, Luni. The sequence listing filed with the application follows.

SEQUENCE LISTING (1 sequence)

SEQ ID NO: 1 - protein, 84 aa, Artificial Sequence
  Synthetic Polypeptide
QGIREVILCKDQDGKIGLRLKSIDNGIFVQLVQANSPASLVGLRFGDQVLQINGENCAGWSSDKAHKVLKQAFGEKITMTIRDR